European Patent Application EP 4 578 877 A1, published July 2, 2025. Title: 靶向FAP和TGFβ的抗体融合蛋白及其用途. Applicant: 南京维立志博生物科技有限公司. The sequence listing filed with the application follows.

SEQUENCE LISTING (45 sequences)

SEQ ID NO: 1 - protein, 113 aa, artificial sequence
DIVMSQSPSSLAVSVGEKVTMSCKSSQSLLYSRNQKNYLAWFQQKPGQSPKLLIFWASTRESGVPDRFTGSGFGTDFNLTISSVQAEDLAVYDCQQYFSYPLTFGAGTKLELK

SEQ ID NO: 2 - protein, 107 aa, artificial sequence [sequence omitted]

SEQ ID NO: 3 - protein, 220 aa, artificial sequence
DIVMSQSPSSLAVSVGEKVTMSCKSSQSLLYSRNQKNYLAWFQQKPGQSPKLLIFWASTRESGVPDRFTGSGFGTDFNLTISSVQAEDLAVYDCQQYFSYPLTFGAGTKLELKRTVAAPSVFIFPPSDEQLKSGTASVVCLLNNFYPREAKVQWKVDNALQSGNSQESVTEQDSKDSTYSLSSTLTLSKADYEKHKVYACEVTHQGLSSPVTKSFNRGEC

SEQ ID NO: 4 - protein, 17 aa, artificial sequence
KSSQSLLYSRNQKNYLA

SEQ ID NO: 5 - protein, 7 aa, artificial sequence
WASTRES

SEQ ID NO: 6 - protein, 9 aa, artificial sequence
QQYFSYPLT

SEQ ID NO: 7 - protein, 124 aa, artificial sequence
EVQLQQSGPELVKPGASVKMSCKTSRYTFTEYTIHWVRQSHGKSLEWIGGINPNNGIPNYNQKFKGRATLTVGKSSSTAYMELRSLTSEDSAVYFCARRRIAYGYDEGHAMDYWGQGTSVTVSS

SEQ ID NO: 8 - protein, 330 aa, artificial sequence [sequence omitted]

SEQ ID NO: 9 - protein, 454 aa, artificial sequence
EVQLQQSGPELVKPGASVKMSCKTSRYTFTEYTIHWVRQSHGKSLEWIGGINPNNGIPNYNQKFKGRATLTVGKSSSTAYMELRSLTSEDSAVYFCARRRIAYGYDEGHAMDYWGQGTSVTVSSASTKGPSVFPLAPSSKSTSGGTAALGCLVKDYFPEPVTVSWNSGALTSGVHTFPAVLQSSGLYSLSSVVTVPSSSLGTQTYICNVNHKPSNTKVDKKVEPKSCDKTHTCPPCPAPELLGGPSVFLFPPKPKDTLMISRTPEVTCVVVDVSHEDPEVKFNWYVDGVEVHNAKTKPREEQYNSTYRVVSVLTVLHQDWLNGKEYKCKVSNKALPAPIEKTISKAKGQPREPQVYTLPPSRDELTKNQVSLTCLVKGFYPSDIAVEWESNGQPENNYKTTPPVLDSDGSFFLYSKLTVDKSRWQQGNVFSCSVMHEALHNHYTQKSLSLSPGK

SEQ ID NO: 10 - protein, 5 aa, artificial sequence
EYTIH

SEQ ID NO: 11 - protein, 17 aa, artificial sequence
GINPNNGIPNYNQKFKG

SEQ ID NO: 12 - protein, 15 aa, artificial sequence
RRIAYGYDEGHAMDY

SEQ ID NO: 13 - protein, 124 aa, artificial sequence
QVQLVQSGAEVKKPGASVKVSCKASGYTFTEYTIHWVRQATGQGLEWIGGINPNNGIPNYNQKFKGRATMTVGTSISTAYMELSSLRSEDTAVYFCARRRIAYGYDEGHAMDYWGQGTLVTVSS

SEQ ID NO: 14 - protein, 454 aa, artificial sequence
QVQLVQSGAEVKKPGASVKVSCKASGYTFTEYTIHWVRQATGQGLEWIGGINPNNGIPNYNQKFKGRATMTVGTSISTAYMELSSLRSEDTAVYFCARRRIAYGYDEGHAMDYWGQGTLVTVSSASTKGPSVFPLAPSSKSTSGGTAALGCLVKDYFPEPVTVSWNSGALTSGVHTFPAVLQSSGLYSLSSVVTVPSSSLGTQTYICNVNHKPSNTKVDKKVEPKSCDKTHTCPPCPAPELLGGPSVFLFPPKPKDTLMISRTPEVTCVVVDVSHEDPEVKFNWYVDGVEVHNAKTKPREEQYNSTYRVVSVLTVLHQDWLNGKEYKCKVSNKALPAPIEKTISKAKGQPREPQVYTLPPSRDELTKNQVSLTCLVKGFYPSDIAVEWESNGQPENNYKTTPPVLDSDGSFFLYSKLTVDKSRWQQGNVFSCSVMHEALHNHYTQKSLSLSPGK

SEQ ID NO: 15 - protein, 113 aa, artificial sequence
DIQMTQSPSSLSASVGDRVTITCKSSQSLLYSRNQKNYLAWFQQKPGKAPKLLIFWASTRESGVPSRFTGSGFGTDFTLTISSLQPEDFATYYCQQYFSYPLTFGQGTKLEIK

SEQ ID NO: 16 - protein, 220 aa, artificial sequence
DIQMTQSPSSLSASVGDRVTITCKSSQSLLYSRNQKNYLAWFQQKPGKAPKLLIFWASTRESGVPSRFTGSGFGTDFTLTISSLQPEDFATYYCQQYFSYPLTFGQGTKLEIKRTVAAPSVFIFPPSDEQLKSGTASVVCLLNNFYPREAKVQWKVDNALQSGNSQESVTEQDSKDSTYSLSSTLTLSKADYEKHKVYACEVTHQGLSSPVTKSFNRGEC

SEQ ID NO: 17 - protein, 124 aa, artificial sequence
QVQLVQSGAEVKKPGASVKVSCKTSRYTFTEYTIHWVRQAPGQRLEWIGGINPNNGIPNYNQKFKGRVTITVDTSASTAYMELSSLRSEDTAVYYCARRRIAYGYDEGHAMDYWGQGTLVTVSS

SEQ ID NO: 18 - protein, 454 aa, artificial sequence
QVQLVQSGAEVKKPGASVKVSCKTSRYTFTEYTIHWVRQAPGQRLEWIGGINPNNGIPNYNQKFKGRVTITVDTSASTAYMELSSLRSEDTAVYYCARRRIAYGYDEGHAMDYWGQGTLVTVSSASTKGPSVFPLAPSSKSTSGGTAALGCLVKDYFPEPVTVSWNSGALTSGVHTFPAVLQSSGLYSLSSVVTVPSSSLGTQTYICNVNHKPSNTKVDKKVEPKSCDKTHTCPPCPAPELLGGPSVFLFPPKPKDTLMISRTPEVTCVVVDVSHEDPEVKFNWYVDGVEVHNAKTKPREEQYNSTYRVVSVLTVLHQDWLNGKEYKCKVSNKALPAPIEKTISKAKGQPREPQVYTLPPSRDELTKNQVSLTCLVKGFYPSDIAVEWESNGQPENNYKTTPPVLDSDGSFFLYSKLTVDKSRWQQGNVFSCSVMHEALHNHYTQKSLSLSPGK

SEQ ID NO: 19 - protein, 113 aa, artificial sequence
DIVMTQSPDSLAVSLGERATINCKSSQSLLYSRNQKNYLAWYQQKPGQPPKLLIFWASTRESGVPDRFSGSGFGTDFTLTISSLQAEDVAVYYCQQYFSYPLTFGQGTKVEIK

SEQ ID NO: 20 - protein, 220 aa, artificial sequence
DIVMTQSPDSLAVSLGERATINCKSSQSLLYSRNQKNYLAWYQQKPGQPPKLLIFWASTRESGVPDRFSGSGFGTDFTLTISSLQAEDVAVYYCQQYFSYPLTFGQGTKVEIKRTVAAPSVFIFPPSDEQLKSGTASVVCLLNNFYPREAKVQWKVDNALQSGNSQESVTEQDSKDSTYSLSSTLTLSKADYEKHKVYACEVTHQGLSSPVTKSFNRGEC

SEQ ID NO: 21 - protein, 124 aa, artificial sequence
QVQLVQSGAEVKKPGASVKVSCKASGYTFTEYTIHWVRQATGQGLEWIGGINPNNRIPNYNQKFKGRATMTVGTSISTAYMELSSLRSEDTAVYFCARRRIAYGYDEGHAMDYWGQGTLVTVSS

SEQ ID NO: 22 - protein, 17 aa, artificial sequence
GINPNNRIPNYNQKFKG

SEQ ID NO: 23 - protein, 454 aa, artificial sequence
QVQLVQSGAEVKKPGASVKVSCKASGYTFTEYTIHWVRQATGQGLEWIGGINPNNRIPNYNQKFKGRATMTVGTSISTAYMELSSLRSEDTAVYFCARRRIAYGYDEGHAMDYWGQGTLVTVSSASTKGPSVFPLAPSSKSTSGGTAALGCLVKDYFPEPVTVSWNSGALTSGVHTFPAVLQSSGLYSLSSVVTVPSSSLGTQTYICNVNHKPSNTKVDKKVEPKSCDKTHTCPPCPAPELLGGPSVFLFPPKPKDTLMISRTPEVTCVVVDVSHEDPEVKFNWYVDGVEVHNAKTKPREEQYNSTYRVVSVLTVLHQDWLNGKEYKCKVSNKALPAPIEKTISKAKGQPREPQVYTLPPSRDELTKNQVSLTCLVKGFYPSDIAVEWESNGQPENNYKTTPPVLDSDGSFFLYSKLTVDKSRWQQGNVFSCSVMHEALHNHYTQKSLSLSPGK

SEQ ID NO: 24 - protein, 136 aa, artificial sequence
IPPHVQKSVNNDMIVTDNNGAVKFPQLCKFCDVRFSTCDNQKSCMSNCSITSICEKPQEVCVAVWRKNDENITLETVCHDPKLPYHDFILEDAASPKCIMKEKKKPGETFFMCSCSSDECNDNIIFSEEYNTSNPD

SEQ ID NO: 25 - protein, 590 aa, artificial sequence
QVQLVQSGAEVKKPGASVKVSCKASGYTFTEYTIHWVRQATGQGLEWIGGINPNNRIPNYNQKFKGRATMTVGTSISTAYMELSSLRSEDTAVYFCARRRIAYGYDEGHAMDYWGQGTLVTVSSASTKGPSVFPLAPSSKSTSGGTAALGCLVKDYFPEPVTVSWNSGALTSGVHTFPAVLQSSGLYSLSSVVTVPSSSLGTQTYICNVNHKPSNTKVDKKVEPKSCDKTHTCPPCPAPELLGGPSVFLFPPKPKDTLMISRTPEVTCVVVDVSHEDPEVKFNWYVDGVEVHNAKTKPREEQYNSTYRVVSVLTVLHQDWLNGKEYKCKVSNKALPAPIEKTISKAKGQPREPQVYTLPPSRDELTKNQVSLTCLVKGFYPSDIAVEWESNGQPENNYKTTPPVLDSDGSFFLYSKLTVDKSRWQQGNVFSCSVMHEALHNHYTQKSLSLSPGAIPPHVQKSVNNDMIVTDNNGAVKFPQLCKFCDVRFSTCDNQKSCMSNCSITSICEKPQEVCVAVWRKNDENITLETVCHDPKLPYHDFILEDAASPKCIMKEKKKPGETFFMCSCSSDECNDNIIFSEEYNTSNPD

SEQ ID NO: 26 - protein, 330 aa, artificial sequence
ASTKGPSVFPLAPSSKSTSGGTAALGCLVKDYFPEPVTVSWNSGALTSGVHTFPAVLQSSGLYSLSSVVTVPSSSLGTQTYICNVNHKPSNTKVDKKVEPKSCDKTHTCPPCPAPELLGGPSVFLFPPKPKDTLMISRTPEVTCVVVDVSHEDPEVKFNWYVDGVEVHNAKTKPREEQYNSTYRVVSVLTVLHQDWLNGKEYKCKVSNKALPAPIEKTISKAKGQPREPQVYTLPPSRDELTKNQVSLTCLVKGFYPSDIAVEWESNGQPENNYKTTPPVLDSDGSFFLYSKLTVDKSRWQQGNVFSCSVMHEALHNHYTQKSLSLSPGA

SEQ ID NO: 27 - protein, 108 aa, artificial sequence
EIVLTQSPGTLSLSPGERATLSCRASQSVSRSYLAWYQQKPGQAPRLLIIGASTRATGIPDRFSGSGSGTDFTLTISRLEPEDFAVYYCQQGQVIPPTFGQGTKVEIK

SEQ ID NO: 28 - protein, 215 aa, artificial sequence
EIVLTQSPGTLSLSPGERATLSCRASQSVSRSYLAWYQQKPGQAPRLLIIGASTRATGIPDRFSGSGSGTDFTLTISRLEPEDFAVYYCQQGQVIPPTFGQGTKVEIKRTVAAPSVFIFPPSDEQLKSGTASVVCLLNNFYPREAKVQWKVDNALQSGNSQESVTEQDSKDSTYSLSSTLTLSKADYEKHKVYACEVTHQGLSSPVTKSFNRGEC

SEQ ID NO: 29 - protein, 582 aa, artificial sequence
EVQLLESGGGLVQPGGSLRLSCAASGFTFSSHAMSWVRQAPGKGLEWVSAIWASGEQYYADSVKGRFTISRDNSKNTLYLQMNSLRAEDTAVYYCAKGWLGNFDYWGQGTLVTVSSASTKGPSVFPLAPSSKSTSGGTAALGCLVKDYFPEPVTVSWNSGALTSGVHTFPAVLQSSGLYSLSSVVTVPSSSLGTQTYICNVNHKPSNTKVDKKVEPKSCDKTHTCPPCPAPELLGGPSVFLFPPKPKDTLMISRTPEVTCVVVDVSHEDPEVKFNWYVDGVEVHNAKTKPREEQYNSTYRVVSVLTVLHQDWLNGKEYKCKVSNKALPAPIEKTISKAKGQPREPQVYTLPPSRDELTKNQVSLTCLVKGFYPSDIAVEWESNGQPENNYKTTPPVLDSDGSFFLYSKLTVDKSRWQQGNVFSCSVMHEALHNHYTQKSLSLSPGAIPPHVQKSVNNDMIVTDNNGAVKFPQLCKFCDVRFSTCDNQKSCMSNCSITSICEKPQEVCVAVWRKNDENITLETVCHDPKLPYHDFILEDAASPKCIMKEKKKPGETFFMCSCSSDECNDNIIFSEEYNTSNPD

SEQ ID NO: 30 - protein, 116 aa, artificial sequence
EVQLLESGGGLVQPGGSLRLSCAASGFTFSSHAMSWVRQAPGKGLEWVSAIWASGEQYYADSVKGRFTISRDNSKNTLYLQMNSLRAEDTAVYYCAKGWLGNFDYWGQGTLVTVSS

SEQ ID NO: 31 - protein, 760 aa, artificial sequence
MKTWVKIVFGVATSAVLALLVMCIVLRPSRVHNSEENTMRALTLKDILNGTFSYKTFFPNWISGQEYLHQSADNNIVLYNIETGQSYTILSNRTMKSVNASNYGLSPDRQFVYLESDYSKLWRYSYTATYYIYDLSNGEFVRGNELPRPIQYLCWSPVGSKLAYVYQNNIYLKQRPGDPPFQITFNGRENKIFNGIPDWVYEEEMLATKYALWWSPNGKFLAYAEFNDTDIPVIAYSYYGDEQYPRTINIPYPKAGAKNPVVRIFIIDTTYPAYVGPQEVPVPAMIASSDYYFSWLTWVTDERVCLQWLKRVQNVSVLSICDFREDWQTWDCPKTQEHIEESRTGWAGGFFVSTPVFSYDAISYYKIFSDKDGYKHIHYIKDTVENAIQITSGKWEAINIFRVTQDSLFYSSNEFEEYPGRRNIYRISIGSYPPSKKCVTCHLRKERCQYYTASFSDYAKYYALVCYGPGIPISTLHDGRTDQEIKILEENKELENALKNIQLPKEEIKKLEVDEITLWYKMILPPQFDRSKKYPLLIQVYGGPCSQSVRSVFAVNWISYLASKEGMVIALVDGRGTAFQGDKLLYAVYRKLGVYEVEDQITAVRKFIEMGFIDEKRIAIWGWSYGGYVSSLALASGTGLFKCGIAVAPVSSWEYYASVYTERFMGLPTKDDNLEHYKNSTVMARAEYFRNVDYLLIHGTADDNVHFQNSAQIAKALVNAQVDFQAMWYSDQNHGLSGLSTNHLYTHMTHFLKQCFSLSD

SEQ ID NO: 32 - protein, 760 aa, artificial sequence
MKTWVKIVFGVATSAVLALLVMCIVLRPPRVHNSEENTMRALTLKDILNGTFSYKTFFPNWISGQEYLHQSADNNIVLYNIETGQSYTILSNRTMKSVNASNYGLSPDRQFVYLESDYSKLWRYSYTATYYIYDLSNGEFVRGNELPRPIQYLCWSPVGSKLAYVYQNNIYLKQRPGDPPFQITFNGRENKIFNGIPDWVYEEEMLATKYALWWSPNGKFLAYAEFNDTDIPVIAYSYYGDEQYPRTINIPYPKAGAKNPFVRIFIIDTTYPAYVGPQEVPVPAMIASSDYYFSWLTWVTDERVCLQWLKRVQNVSVLSICDFREDWQTWDCPKTQEHIEESRTGWAGGFFVSTPVFSYDAISYYKIFSDKDGYKHIHYIKDTVENAIQITSGKWEAINIFRVTQDSLFYSSNEFEDYPGRRNIYRISIGSYPPSKKCVTCHLRKERCQYYTASFSDYAKYYALVCYGPGIPISTLHDGRTDQEIKILEENKELENALKNIQLPKEEIKKLEVDEITLWYKMILPPQFDRSKKYPLLIQVYGGPCSQSVRSVFAVNWISYLASKEGMVIALVDGRGTAFQGDKLLYAVYRKLGVYEVEDQITAVRKFIEMGFIDEKRIAIWGWSYGGYVSSLALASGTGLFKCGIAVAPVSSWEYYASVYTERFMGLPTKDDNLEHYKNSTVMARAEYFRNVDYLLIHGTADDNVHFQNSAQIAKALVNAQVDFQAMWYSDQNHGLSGLSTNHLYTHMTHFLKQCFSLSD

SEQ ID NO: 33 - protein, 766 aa, artificial sequence
MKTPWKVLLGLLGAAALVTIITVPVVLLNKGTDDATADSRKTYTLTDYLKNTYRLKLYSLRWISDHEYLYKQENNILVFNAEYGNSSVFLENSTFDEFGHSINDYSISPDGQFILLEYNYVKQWRHSYTASYDIYDLNKRQLITEERIPNNTQWVTWSPVGHKLAYVWNNDIYVKIEPNLPSYRITWTGKEDIIYNGITDWVYEEEVFSAYSALWWSPNGTFLAYAQFNDTEVPLIEYSFYSDESLQYPKTVRVPYPKAGAVNPTVKFFVVNTDSLSSVTNATSIQITAPASMLIGDHYLCDVTWATQERISLQWLRRIQNYSVMDICDYDESSGRWNCLVARQHIEMSTTGWVGRFRPSEPHFTLDGNSFYKIISNEEGYRHICYFQIDKKDCTFITKGTWEVIGIEALTSDYLYYISNEYKGMPGGRNLYKIQLSDYTKVTCLSCELNPERCQYYSVSFSKEAKYYQLRCSGPGLPLYTLHSSVNDKGLRVLEDNSALDKMLQNVQMPSKKLDFIILNETKFWYQMILPPHFDKSKKYPLLLDVYAGPCSQKADTVFRLNWATYLASTENIIVASFDGRGSGYQGDKIMHAINRRLGTFEVEDQIEAARQFSKMGFVDNKRIAIWGWSYGGYVTSMVLGSGSGVFKCGIAVAPVSRWEYYDSVYTERYMGLPTPEDNLDHYRNSTVMSRAENFKQVEYLLIHGTADDNVHFQQSAQISKALVDVGVDFQAMWYTDEDHGIASSTAHQHIYTHMSHFIKQCFSLP

SEQ ID NO: 34 - protein, 544 aa, artificial sequence
IPPHVQKSVNNDMIVTDNNGAVKFPQLCKFCDVRFSTCDNQKSCMSNCSITSICEKPQEVCVAVWRKNDENITLETVCHDPKLPYHDFILEDAASPKCIMKEKKKPGETFFMCSCSSDECNDNIIFSEEYNTSNPDLLLVIFQVTGISLLPPLGVAISVIIIFYCYRVNRQQKLSSTWETGKTRKLMEFSEHCAIILEDDRSDISSTCANNINHNTELLPIELDTLVGKGRFAEVYKAKLKQNTSEQFETVAVKIFPYEEYASWKTEKDIFSDINLKHENILQFLTAEERKTELGKQYWLITAFHAKGNLQEYLTRHVISWEDLRKLGSSLARGIAHLHSDHTPCGRPKMPIVHRDLKSSNILVKNDLTCCLCDFGLSLRLDPTLSVDDLANSGQVGTARYMAPEVLESRMNLENVESFKQTDVYSMALVLWEMTSRCNAVGEVKDYEPPFGSKVREHPCVESMKDNVLRDRGRPEIPSFWLNHQGIQMVCETLTECWDHDPEARLTAQCVAERFSELEHLDRLSGRSCSEEKIPEDGSLNTTK

SEQ ID NO: 35 - protein, 454 aa, artificial sequence
QVQLVQSGAEVKKPGASVKVSCKASGYTFTEYTIHWVRQATGQGLEWIGGINPNNRIPNYNQKFKGRATMTVGTSISTAYMELSSLRSEDTAVYFCARRRIAYGYDEGHAMDYWGQGTLVTVSSASTKGPSVFPLAPSSKSTSGGTAALGCLVKDYFPEPVTVSWNSGALTSGVHTFPAVLQSSGLYSLSSVVTVPSSSLGTQTYICNVNHKPSNTKVDKKVEPKSCDKTHTCPPCPAPELLGGPSVFLFPPKPKDTLMISRTPEVTCVVVDVSHEDPEVKFNWYVDGVEVHNAKTKPREEQYNSTYRVVSVLTVLHQDWLNGKEYKCKVSNKALPAPIEKTISKAKGQPREPQVYTLPPSRDELTKNQVSLTCLVKGFYPSDIAVEWESNGQPENNYKTTPPVLDSDGSFFLYSKLTVDKSRWQQGNVFSCSVMHEALHNHYTQKSLSLSPGA

SEQ ID NO: 36 - protein, 610 aa, artificial sequence
QVQLVQSGAEVKKPGASVKVSCKASGYTFTEYTIHWVRQATGQGLEWIGGINPNNRIPNYNQKFKGRATMTVGTSISTAYMELSSLRSEDTAVYFCARRRIAYGYDEGHAMDYWGQGTLVTVSSASTKGPSVFPLAPSSKSTSGGTAALGCLVKDYFPEPVTVSWNSGALTSGVHTFPAVLQSSGLYSLSSVVTVPSSSLGTQTYICNVNHKPSNTKVDKKVEPKSCDKTHTCPPCPAPELLGGPSVFLFPPKPKDTLMISRTPEVTCVVVDVSHEDPEVKFNWYVDGVEVHNAKTKPREEQYNSTYRVVSVLTVLHQDWLNGKEYKCKVSNKALPAPIEKTISKAKGQPREPQVYTLPPSRDELTKNQVSLTCLVKGFYPSDIAVEWESNGQPENNYKTTPPVLDSDGSFFLYSKLTVDKSRWQQGNVFSCSVMHEALHNHYTQKSLSLSPGAGGGGSGGGGSGGGGSGGGGSIPPHVQKSVNNDMIVTDNNTAVKFPQLCKFCDVRFSTCDNQKSCMSNCSITSICEKPQEVCVAVWRKNDENITLETVCHDPKLPYHDFILEDAASPKCIMKEKKKPGETFFMCSCSSDECNDNIIFSEEYNTSNPD

SEQ ID NO: 37 - protein, 136 aa, artificial sequence
IPPHVQKSVNNDMIVTDNNTAVKFPQLCKFCDVRFSTCDNQKSCMSNCSITSICEKPQEVCVAVWRKNDENITLETVCHDPKLPYHDFILEDAASPKCIMKEKKKPGETFFMCSCSSDECNDNIIFSEEYNTSNPD

SEQ ID NO: 38 - protein, 610 aa, artificial sequence
QVQLVQSGAEVKKPGASVKVSCKASGYTFTEYTIHWVRQATGQGLEWIGGINPNNRIPNYNQKFKGRATMTVGTSISTAYMELSSLRSEDTAVYFCARRRIAYGYDEGHAMDYWGQGTLVTVSSASTKGPSVFPLAPSSKSTSGGTAALGCLVKDYFPEPVTVSWNSGALTSGVHTFPAVLQSSGLYSLSSVVTVPSSSLGTQTYICNVNHKPSNTKVDKKVEPKSCDKTHTCPPCPAPELLGGPSVFLFPPKPKDTLMISRTPEVTCVVVDVSHEDPEVKFNWYVDGVEVHNAKTKPREEQYNSTYRVVSVLTVLHQDWLNGKEYKCKVSNKALPAPIEKTISKAKGQPREPQVYTLPPSRDELTKNQVSLTCLVKGFYPSDIAVEWESNGQPENNYKTTPPVLDSDGSFFLYSKLTVDKSRWQQGNVFSCSVMHEALHNHYTQKSLSLSPGAGGGGSGGGGSGGGGSGGGGSIPPHVQKSVNNDMIVTDNEGAVKFPQLCKFCDVRFSTCDNQKSCMSNCSITSICEKPQEVCVAVWRKNDENITLETVCHDPKLPYHDFILEDAASPKCIMKEKKKPGETFFMCSCSSDECNDNIIFSEEYNTSNPD

SEQ ID NO: 39 - protein, 136 aa, artificial sequence
IPPHVQKSVNNDMIVTDNEGAVKFPQLCKFCDVRFSTCDNQKSCMSNCSITSICEKPQEVCVAVWRKNDENITLETVCHDPKLPYHDFILEDAASPKCIMKEKKKPGETFFMCSCSSDECNDNIIFSEEYNTSNPD

SEQ ID NO: 40 - protein, 232 aa, artificial sequence
EPKSCDKTHTCPPCPAPELLGGPSVFLFPPKPKDTLMISRTPEVTCVVVDVSHEDPEVKFNWYVDGVEVHNAKTKPREEQYNSTYRVVSVLTVLHQDWLNGKEYKCKVSNKALPAPIEKTISKAKGQPREPQVYTLPPSRDELTKNQVSLTCLVKGFYPSDIAVEWESNGQPENNYKTTPPVLDSDGSFFLYSKLTVDKSRWQQGNVFSCSVMHEALHNHYTQKSLSLSPGK

SEQ ID NO: 41 - protein, 446 aa, artificial sequence
EVQLLESGGGLVQPGGSLRLSCAASGFTFSSHAMSWVRQAPGKGLEWVSAIWASGEQYYADSVKGRFTISRDNSKNTLYLQMNSLRAEDTAVYYCAKGWLGNFDYWGQGTLVTVSSASTKGPSVFPLAPSSKSTSGGTAALGCLVKDYFPEPVTVSWNSGALTSGVHTFPAVLQSSGLYSLSSVVTVPSSSLGTQTYICNVNHKPSNTKVDKKVEPKSCDKTHTCPPCPAPELLGGPSVFLFPPKPKDTLMISRTPEVTCVVVDVSHEDPEVKFNWYVDGVEVHNAKTKPREEQYNSTYRVVSVLTVLHQDWLNGKEYKCKVSNKALPAPIEKTISKAKGQPREPQVYTLPPSRDELTKNQVSLTCLVKGFYPSDIAVEWESNGQPENNYKTTPPVLDSDGSFFLYSKLTVDKSRWQQGNVFSCSVMHEALHNHYTQKSLSLSPGA

SEQ ID NO: 42 - protein, 446 aa, artificial sequence
EVQLLESGGGLVQPGGSLRLSCAASGFTFSSHAMSWVRQAPGKGLEWVSAIWASGEQYYADSVKGRFTISRDNSKNTLYLQMNSLRAEDTAVYYCAKGWLGNFDYWGQGTLVTVSSASTKGPSVFPLAPSSKSTSGGTAALGCLVKDYFPEPVTVSWNSGALTSGVHTFPAVLQSSGLYSLSSVVTVPSSSLGTQTYICNVNHKPSNTKVDKKVEPKSCDKTHTCPPCPAPELLGGPSVFLFPPKPKDTLMISRTPEVTCVVVDVSHEDPEVKFNWYVDGVEVHNAKTKPREEQYNSTYRVVSVLTVLHQDWLNGKEYKCKVSNKALPAPIEKTISKAKGQPREPQVYTLPPSRDELTKNQVSLTCLVKGFYPSDIAVEWESNGQPENNYKTTPPVLDSDGSFFLYSKLTVDKSRWQQGNVFSCSVMHEALHNHYTQKSLSLSPGK

SEQ ID NO: 43 - protein, 5 aa, artificial sequence
  REPEAT 1..5: note = REPEAT=1-10, e.g., 1, 2, 3, 4, 5 or 6
GGGGS

SEQ ID NO: 44 - protein, 5 aa, artificial sequence
EPKSC

SEQ ID NO: 45 - protein, 5 aa, artificial sequence
EPKSS